European Patent Application EP 4 215 245 A1, published July 26, 2023. Title: Enhanced Chimeric Antigen Receptor Cells in Hypoxic Tumor Microenvironment. Applicant: Innovative Cellular Therapeutics Holdings, Ltd. Application US. The sequence listing filed with the application follows.

SEQUENCE LISTING (27 sequences)

SEQ ID NO: 1 - DNA, 306 bp, Homo sapiens
  source 1..306: mol_type = genomic DNA
ggccctacgtgctgtctcacacagcctgtctgacggccctacgtgctgtctcacacagcctgtctgacggccctacgtgctgtctcacacagcctgtctgacggccctacgtgctgtctcacacagcctgtctgacggccctacgtgctgtctcacacagcctgtctgacggccctacgtgctgtctcacacagcctgtctgacggccctacgtgctgtctcacacagcctgtctgacggccctacgtgctgtctcacacagcctgtctgacggccctacgtgctgtctcacacagcctgtctgac

SEQ ID NO: 2 - DNA, 113 bp, Homo sapiens
  source 1..113: mol_type = genomic DNA
cattttgacacccccataatatttttccagaattaacagtataaattgcatctcttgttcaagagttccctatcactctctttaatcactactcacagtaacctcaactcctg

SEQ ID NO: 3 - DNA, 63 bp, Homo sapiens
  source 1..63: mol_type = genomic DNA
atggcgctgccggtgaccgcgctgttactgccgctggcgctgttactgcacgccgcgcgcccg

SEQ ID NO: 4 - protein, 21 aa, Homo sapiens
MALPVTALLLPLALLLHAARP

SEQ ID NO: 5 - DNA, 735 bp, synthetic construct
  source 1..735: mol_type = other DNA
gaaatcgtgctgacgcagagtccggcgaccctgagcttaagcccgggcgaacgcgcgacgctgagctgccgcgcgagcgaaagcgtggataactatggcctgagctttattaactggtttcagcagaaaccgggccaagcgccgcgcctgctgatttatggcacgagcaaccgcggcagcggcattccggcgcgctttagcggcagcggtagtggcaccgattttaccctgaccattagcagcctggaaccggaagattttgcggtgtatttttgtcagcagagcaacgaagtgccgtatacctttggcggtggcaccaaagtggaaattaaaggcggtggtggtagcggtggtggcggtagcggcggcggtggcagccaagtgcagctggtgcagagcggcgcggaagtgaaaaaaccgggcgcgagcgtgaaagtgagctgcaaagcgagcggctataccctgaccgattataacatggattgggtgcgccaagcgccgggccaaggcctggaatggattggcgatatttatccgaacaccggcggcaccatttataatcagaaatttaaaggccgcgtgaccatgaccattgatacgagcacgagcaccgtgtatatggaactgagcagcctgcgcagcgaagataccgcggtgtattattgcacccgctttcgcggcattcattatgcgatggattattggggccaaggcaccaccgtgaccgtgagcagc

SEQ ID NO: 6 - protein, 245 aa, synthetic construct
EIVLTQSPATLSLSPGERATLSCRASESVDNYGLSFINWFQQKPGQAPRLLIYGTSNRGSGIPARFSGSGSGTDFTLTISSLEPEDFAVYFCQQSNEVPYTFGGGTKVEIKGGGGSGGGGSGGGGSQVQLVQSGAEVKKPGASVKVSCKASGYTLTDYNMDWVRQAPGQGLEWIGDIYPNTGGTIYNQKFKGRVTMTIDTSTSTVYMELSSLRSEDTAVYYCTRFRGIHYAMDYWGQGTTVTVSS

SEQ ID NO: 7 - DNA, 669 bp, Homo sapiens
  source 1..669: mol_type = genomic DNA
accacgacgccagcgccgcgaccaccaacaccggcgcccaccatcgcgtcgcagcccctgtccctgcgcccagaggcgtgccggccagcggcggggggcgcagtgcacacgagggggctggacttcgcctgtgatatctacatctgggcgcccttggccgggacttgtggggtccttctcctgtcactggttatcaccctttactgcaaacggggcagaaagaaactcctgtatatattcaaacaaccatttatgagaccagtacaaactactcaagaggaagatggctgtagctgccgatttccagaagaagaagaaggaggatgtgaactgagagtgaagttcagcaggagcgcagacgcccccgcgtaccagcagggccagaaccagctctataacgagctcaatctaggacgaagagaggagtacgatgttttggacaagaggcgtggccgggaccctgagatggggggaaagccgagaaggaagaaccctcaggaaggcctgtacaatgaactgcagaaagataagatggcggaggcctacagtgagattgggatgaaaggcgagcgccggaggggcaaggggcacgatggcctttaccagggtctcagtacagccaccaaggacacctacgacgcccttcacatgcaggccctgccccctcgc

SEQ ID NO: 8 - protein, 223 aa, Homo sapiens
TTTPAPRPPTPAPTIASQPLSLRPEACRPAAGGAVHTRGLDFACDIYIWAPLAGTCGVLLLSLVITLYCKRGRKKLLYIFKQPFMRPVQTTQEEDGCSCRFPEEEEGGCELRVKFSRSADAPAYQQGQNQLYNELNLGRREEYDVLDKRRGRDPEMGGKPRRKNPQEGLYNELQKDKMAEAYSEIGMKGERRRGKGHDGLYQGLSTATKDTYDALHMQALPPR

SEQ ID NO: 9 - DNA, 612 bp, Homo sapiens
  source 1..612: mol_type = genomic DNA
gcgccggcggcgggcgataccattattagcctggattttggcagcaacgataccgaaaccgatgatcagcagctggaagaagtgccgctgtataacgatgtgatgctgccgagcccgaacgaaaaactgcagaacattaacctggcgatgagcccgctgccaacggccgaaaccccgaaaccgttacgcagcagcgcggatccggcgctgaaccaagaagtggcgctgaaactggaaccgaacccggaaagcctggaactgagctttaccatgccgcagattcaagatcagaccccgagcccgagcgatggcagcacccgtcagagcagcccggaaccgaacagcccgagcgaatattgcttttatgtggatagcgatatggtgaacgaatttaaactggaactggtggaaaaactgtttgcggaagataccgaagcgaaaaacccgtttagcacccaagataccgatctggatctggaaatgctggcgccgtatattccgatggatgacgattttcagctgcgcagctttgatcagctgagcccgctggaaagcagcagtgcgagcccggaaagcgcgagcccgcagagcaccgtgaccgtgtttcagtaa

SEQ ID NO: 10 - protein, 203 aa, Homo sapiens
APAAGDTIISLDFGSNDTETDDQQLEEVPLYNDVMLPSPNEKLQNINLAMSPLPTAETPKPLRSSADPALNQEVALKLEPNPESLELSFTMPQIQDQTPSPSDGSTRQSSPEPNSPSEYCFYVDSDMVNEFKLELVEKLFAEDTEAKNPFSTQDTDLDLEMLAPYIPMDDDFQLRSFDQLSPLESSSASPESASPQSTVTVFQ

SEQ ID NO: 11 - DNA, 170 bp, synthetic construct
  source 1..170: mol_type = other DNA
ggccctacgtgctgtctcacacagcctgtctgacggccctacgtgctgtctcacacagcctgtctgacggccctacgtgctgtctcacacagcctgtctgacggccctacgtgctgtctcacacagcctgtctgacggccctacgtgctgtctcacacagcctgtctgac

SEQ ID NO: 12 - DNA, 175 bp, synthetic construct
  source 1..175: mol_type = other DNA
ccacagtgcatacgtgggctccaacaggtcctcttccacagtgcatacgtgggctccaacaggtcctcttccacagtgcatacgtgggctccaacaggtcctcttccacagtgcatacgtgggctccaacaggtcctcttccacagtgcatacgtgggctccaacaggtcctctt

SEQ ID NO: 13 - DNA, 212 bp, Homo sapiens
  source 1..212: mol_type = genomic DNA
gggcagagcgcacatcgcccacagtccccgagaagttggggggaggggtcggcaattgaaccggtgcctagagaaggtggcgcggggtaaactgggaaagtgatgtcgtgtactggctccgcctttttcccgagggtgggggagaaccgtatataagtgcagtagtcgccgtgaacgttctttttcgcaacgggtttgccgccagaacacag

SEQ ID NO: 14 - protein, 240 aa, synthetic construct
EIVLTQSPGTLSLSPGERATLSCRASQSVTSSYLAWYQQKPGQAPRLLINVGSRRATGIPDRFSGSGSGTDFTLTISRLEPEDFAVYYCQQGIMLPPTFGQGTKVEIKGGGGSGGGGSGGGGSEVQLLESGGGLVQPGGSLRLSCAASGFTFSSYAMSWVRQAPGKGLEWVSAIIGSGASTYYADSVKGRFTISRDNSKNTLYLQMNSLRAEDTAVYYCAKGWFGGFNYWGQGTLVTVSS

SEQ ID NO: 15 - DNA, 30 bp, Homo sapiens
  source 1..30: mol_type = genomic DNA
gaagcagctgctagaaaagccgctgccaga

SEQ ID NO: 16 - DNA, 162 bp, synthetic construct
  source 1..162: mol_type = other DNA
ttggacttagagatgttggctccctatatccccatggatgacgattttcagctgctggacctggaaatgcttgccccctacatccctatggatgacgactttcagctgctggacctggagatgctcgccccttacatcccgatggacgatgatttccaactc

SEQ ID NO: 17 - protein, 54 aa, synthetic construct
LDLEMLAPYIPMDDDFQLLDLEMLAPYIPMDDDFQLLDLEMLAPYIPMDDDFQL

SEQ ID NO: 18 - DNA, 108 bp, Homo sapiens
  source 1..108: mol_type = genomic DNA
ttggacttagagatgttggctccctatatccccatggatgacgattttcagctgctggacctggaaatgcttgccccctacatccctatggatgacgactttcagctg

SEQ ID NO: 19 - protein, 36 aa, Homo sapiens
LDLEMLAPYIPMDDDFQLLDLEMLAPYIPMDDDFQL

SEQ ID NO: 20 - DNA, 738 bp, synthetic construct
  source 1..738: mol_type = other DNA
gacatcgtgatgacccagtcccccagctctttaacagtcaccgccggagagaaggtgaccatgagctgcaagtcctcccagtctttactgaacagcggcaaccagaagaactatttaacatggtaccagcagaagcccggtcagccccccaagttattaatctactgggccagcacaagggagagcggcgtgcccgatagattcaccggcagcggctccggcaccgacttcacactgaccatctccagcgtgcaagctgaggatttagccgtgtactactgccagaacgactacagctaccccttcaccttcggcagcggcaccaagctggagattaagggcggcggcggaagcggaggaggaggctccggaggaggaggatcccaagttcagctgcagcagcccggtgccgaactggttcgtcccggtgccagcgtgaagctgagctgcaaggcctccggctacaccttcaccagctactggatcaactgggtgaagcaacgtcccggtcaaggcttagaatggatcggcaacatctaccccagcgactcctacaccaactacaaccagaagttcaaggacaaggccaccctcaccgtggataagagctccagcacagcctacatgcagctgagcagccccacctccgaggatagcgccgtgtattactgtacaaggagctggagaggcaacagctttgactactggggccaaggtacaactttaaccgtgtccagc

SEQ ID NO: 21 - protein, 246 aa, synthetic construct
DIVMTQSPSSLTVTAGEKVTMSCKSSQSLLNSGNQKNYLTWYQQKPGQPPKLLIYWASTRESGVPDRFTGSGSGTDFTLTISSVQAEDLAVYYCQNDYSYPFTFGSGTKLEIKGGGGSGGGGSGGGGSQVQLQQPGAELVRPGASVKLSCKASGYTFTSYWINWVKQRPGQGLEWIGNIYPSDSYTNYNQKFKDKATLTVDKSSSTAYMQLSSPTSEDSAVYYCTRSWRGNSFDYWGQGTTLTVSS

SEQ ID NO: 22 - DNA, 726 bp, synthetic construct
  source 1..726: mol_type = other DNA
gatgtggtgatgacgcagagcccgttaagcctgccggtgaccccgggcgaaccggcgagcattagctgccgcagcagtcagagcctggtgcatagcaacgcgaacacctatctgcattggtatctgcagaaaccgggtcagagcccgcagctgctgatttataaagtgagcaaccgctttagcggcgtgccggatcgcttcagcggcagcggtagcggcaccgattttaccctgaaaattagccgcgtggaagcggaagatgtgggcgtgtattattgcagtcagaacacccatgtgccgccgacctttggtcaaggcacgaaactggaaattaaaggcggtggcggcagcggcggtggcggcagcggtggcggtggcagtcaagtgcagctggtgcagagcggcgcggaagtgaaaaaaccgggcgcgagcgtgaaagtgagctgcaaagcgagcggctatacctttaccgattatgaaatgcattgggtgcgccaagcgccgggccaaggcctggaatggatgggcgcgctggatccgaaaaccggcgataccgcgtatagtcagaaatttaaaggccgcgtgaccctgaccgcggatgaaagcacgagcaccgcgtatatggaactgagcagcctgcgcagcgaagataccgcggtttattattgcacgcgcttttatagctatacctattggggccaaggcacgttagtgaccgtgagcagc

SEQ ID NO: 23 - protein, 242 aa, synthetic construct
DVVMTQSPLSLPVTPGEPASISCRSSQSLVHSNANTYLHWYLQKPGQSPQLLIYKVSNRFSGVPDRFSGSGSGTDFTLKISRVEAEDVGVYYCSQNTHVPPTFGQGTKLEIKGGGGSGGGGSGGGGSQVQLVQSGAEVKKPGASVKVSCKASGYTFTDYEMHWVRQAPGQGLEWMGALDPKTGDTAYSQKFKGRVTLTADESTSTAYMELSSLRSEDTAVYYCTRFYSYTYWGQGTLVTVSS

SEQ ID NO: 24 - protein, 15 aa, synthetic construct
GGGGSGGGGSGGGGS

SEQ ID NO: 25 - protein, 241 aa, synthetic construct
EIVMTQSPATLSVSPGERATLSCRASQSVSRNLAWYQQKPGQAPRLLIYGASTRATGIPARFSGSGSGTEFTLTIGSLQSEDFAVYYCQQYKTWPRTFGQGTNVEIKGGGGSGGGGSGGGGSQVQLQQWGAGLLKPSETLSLTCAVFGGSFSGYYWSWIRQPPGKGLEWIGEINHRGNTNDNPSLKSRVTISVDTSKNQFALKLSSVTAADTAVYYCARERGYTYGNFDHWGQGTLVTVSS

SEQ ID NO: 26 - DNA, 54 bp, Homo sapiens
  source 1..54: mol_type = genomic DNA
ttggacttagagatgttggctccctatatccccatggatgacgattttcagctg

SEQ ID NO: 27 - protein, 18 aa, Homo sapiens
LDLEMLAPYIPMDDDFQL